European Patent Specification EP 3 893 900 B1, published November 5, 2025. Title: NRF-2 DEFICIENT CELLS AND USES THEREOF. Applicant: PUSAN NATIONAL UNIVERSITY INDUSTRY-UNIVERSITY COOPERATION FOUNDATION NEOIMMUNETECH, INC. The sequence listing filed with the application follows.

SEQUENCE LISTING (6 sequences)

SEQ ID NO: 1 - protein, 605 aa, Homo sapiens
MMDLELPPPGLPSQQDMDLIDILWRQDIDLGVSREVFDFSQRRKEYELEKQKKLEKERQEQLQKEQEKAFFAQLQLDEETGEFLPIQPAQHIQSETSGSANYSQVAHIPKSDALYFDDCMQLLAQTFPFVDDNEVSSATFQSLVPDIPGHIESPVFIATNQAQSPETSVAQVAPVDLDGMQQDIEQVWEELLSIPELQCLNIENDKLVETTMVPSPEAKLTEVDNYHFYSSIPSMEKEVGNCSPHFLNAFEDSFSSILSTEDPNQLTVNSLNSDATVNTDFGDEFYSAFIAEPSISNSMPSPATLSHSLSELLNGPIDVSDLSLCKAFNQNHPESTAEFNDSDSGISLNTSPSVASPEHSVESSSYGDTLLGLSDSEVEELDSAPGSVKQNGPKTPVHSSGDMVQPLSPSQGQSTHVHDAQCENTPEKELPVSPGHRKTPFTKDKHSSRLEAHLTRDELRAKALHIPFPVEKIINLPVVDFNEMMSKEQFNEAQLALIRDIRRRGKNKVAAQNCRKRKLENIVELEQDLDHLKDEKEKLLKEKGENDKSLHLLKKQLSTLYLEVFSMLRDEDGKPYSPSEYSLQQTRDGNVFLVPKSKKPDVKKN

SEQ ID NO: 2 - protein, 589 aa, Homo sapiens
MDLIDILWRQDIDLGVSREVFDFSQRRKEYELEKQKKLEKERQEQLQKEQEKAFFAQLQLDEETGEFLPIQPAQHIQSETSGSANYSQVAHIPKSDALYFDDCMQLLAQTFPFVDDNEVSSATFQSLVPDIPGHIESPVFIATNQAQSPETSVAQVAPVDLDGMQQDIEQVWEELLSIPELQCLNIENDKLVETTMVPSPEAKLTEVDNYHFYSSIPSMEKEVGNCSPHFLNAFEDSFSSILSTEDPNQLTVNSLNSDATVNTDFGDEFYSAFIAEPSISNSMPSPATLSHSLSELLNGPIDVSDLSLCKAFNQNHPESTAEFNDSDSGISLNTSPSVASPEHSVESSSYGDTLLGLSDSEVEELDSAPGSVKQNGPKTPVHSSGDMVQPLSPSQGQSTHVHDAQCENTPEKELPVSPGHRKTPFTKDKHSSRLEAHLTRDELRAKALHIPFPVEKIINLPVVDFNEMMSKEQFNEAQLALIRDIRRRGKNKVAAQNCRKRKLENIVELEQDLDHLKDEKEKLLKEKGENDKSLHLLKKQLSTLYLEVFSMLRDEDGKPYSPSEYSLQQTRDGNVFLVPKSKKPDVKKN

SEQ ID NO: 3 - protein, 582 aa, Homo sapiens
MDLIDILWRQDIDLGVSREVFDFSQRRKEYELEKQKKLEKERQEQLQKEQEKAFFAQLQLDEETGEFLPIQPAQHIQSETSGSANYSQVAHIPKSDALYFDDCMQLLAQTFPFVDDNESLVPDIPGHIESPVFIATNQAQSPETSVAQVAPVDLDGMQQDIEQVWEELLSIPELQCLNIENDKLVETTMVPSPEAKLTEVDNYHFYSSIPSMEKEVGNCSPHFLNAFEDSFSSILSTEDPNQLTVNSLNSDATVNTDFGDEFYSAFIAEPSISNSMPSPATLSHSLSELLNGPIDVSDLSLCKAFNQNHPESTAEFNDSDSGISLNTSPSVASPEHSVESSSYGDTLLGLSDSEVEELDSAPGSVKQNGPKTPVHSSGDMVQPLSPSQGQSTHVHDAQCENTPEKELPVSPGHRKTPFTKDKHSSRLEAHLTRDELRAKALHIPFPVEKIINLPVVDFNEMMSKEQFNEAQLALIRDIRRRGKNKVAAQNCRKRKLENIVELEQDLDHLKDEKEKLLKEKGENDKSLHLLKKQLSTLYLEVFSMLRDEDGKPYSPSEYSLQQTRDGNVFLVPKSKKPDVKKN

SEQ ID NO: 4 - DNA, 2446 bp, Homo sapiens
gattaccgagtgccggggagcccggaggagccgccgacgcagccgccaccgccgccgccgccgccaccagagccgccctgtccgcgccgcgcctcggcagccggaacagggccgccgtcggggagccccaacacacggtccacagctcatcatgatggacttggagctgccgccgccgggactcccgtcccagcaggacatggatttgattgacatactttggaggcaagatatagatcttggagtaagtcgagaagtatttgacttcagtcagcgacggaaagagtatgagctggaaaaacagaaaaaacttgaaaaggaaagacaagaacaactccaaaaggagcaagagaaagcctttttcgctcagttacaactagatgaagagacaggtgaatttctcccaattcagccagcccagcacatccagtcagaaaccagtggatctgccaactactcccaggttgcccacattcccaaatcagatgctttgtactttgatgactgcatgcagcttttggcgcagacattcccgtttgtagatgacaatgaggtttcttcggctacgtttcagtcacttgttcctgatattcccggtcacatcgagagcccagtcttcattgctactaatcaggctcagtcacctgaaacttctgttgctcaggtagcccctgttgatttagacggtatgcaacaggacattgagcaagtttgggaggagctattatccattcctgagttacagtgtcttaatattgaaaatgacaagctggttgagactaccatggttccaagtccagaagccaaactgacagaagttgacaattatcatttttactcatctataccctcaatggaaaaagaagtaggtaactgtagtccacattttcttaatgcttttgaggattccttcagcagcatcctctccacagaagaccccaaccagttgacagtgaactcattaaattcagatgccacagtcaacacagattttggtgatgaattttattctgctttcatagctgagcccagtatcagcaacagcatgccctcacctgctactttaagccattcactctctgaacttctaaatgggcccattgatgtttctgatctatcactttgcaaagctttcaaccaaaaccaccctgaaagcacagcagaattcaatgattctgactccggcatttcactaaacacaagtcccagtgtggcatcaccagaacactcagtggaatcttccagctatggagacacactacttggcctcagtgattctgaagtggaagagctagatagtgcccctggaagtgtcaaacagaatggtcctaaaacaccagtacattcttctggggatatggtacaacccttgtcaccatctcaggggcagagcactcacgtgcatgatgcccaatgtgagaacacaccagagaaagaattgcctgtaagtcctggtcatcggaaaaccccattcacaaaagacaaacattcaagccgcttggaggctcatctcacaagagatgaacttagggcaaaagctctccatatcccattccctgtagaaaaaatcattaacctccctgttgttgacttcaacgaaatgatgtccaaagagcagttcaatgaagctcaacttgcattaattcgggatatacgtaggaggggtaagaataaagtggctgctcagaattgcagaaaaagaaaactggaaaatatagtagaactagagcaagatttagatcatttgaaagatgaaaaagaaaaattgctcaaagaaaaaggagaaaatgacaaaagccttcacctactgaaaaaacaactcagcaccttatatctcgaagttttcagcatgctacgtgatgaagatggaaaaccttattctcctagtgaatactccctgcagcaaacaagagatggcaatgttttccttgttcccaaaagtaagaagccagatgttaagaaaaactagatttaggaggatttgaccttttctgagctagtttttttgtactattatactaaaagctcctactgtgatgtgaaatgctcatactttataagtaattctatgcaaaatcatagccaaaactagtatagaaaataatacgaaactttaaaaagcattggagtgtcagtatgttgaatcagtagtttcactttaactgtaaacaatttcttaggacaccatttgggctagtttctgtgtaagtgtaaatactacaaaaacttatttatactgttcttatgtcatttgttatattcatagatttatatgatgatatgacatctggctaaaaagaaattattgcaaaactaaccactatgtacttttttataaatactgtatggacaaaaaatggcattttttatattaaattgtttagctctggcaaaaaaaaaaaattttaagagctggtactaataaaggattattatgactgttaaa

SEQ ID NO: 5 - DNA, 2862 bp, Homo sapiens
ggcccttccggggctgcgcggctcccccgcctcggtgccggcaaaaatgtgcctagtcacggggccgctctcgggggaactgaggtcgccttcgggctgggacccggagccccttcgccgcgccccaagacctccttgagtgcgggctgcgacgcgctcaccccgctgggccgtctgtgggcgcggctttgcgaagtcatccatctctcggatcactctctggcagccttgagctctcttgaaagcccagccccgggacgagggaggagcgccttaagtgcccagcgggctcagaagccccgacgtgtggcggctgagccgggccccgcgcactttctcggccggggaggggttcgggctcgggcacccggagttggcccctcgtaacgccgcgggaaagtgcgggcgagggcagtggactctgaggccggagtcggcggcacccggggcttctagttcggacgcggtgccccctggtggcgctcaccgcgcgcgtggccttggcttccgtgacagcgctcggttggccgtcacagcagccctcggttggccctttcctgctttatagcgtgcaaacctcgccgcgccagggccaagggacaggacatggatttgattgacatactttggaggcaagatatagatcttggagtaagtcgagaagtatttgacttcagtcagcgacggaaagagtatgagctggaaaaacagaaaaaacttgaaaaggaaagacaagaacaactccaaaaggagcaagagaaagcctttttcgctcagttacaactagatgaagagacaggtgaatttctcccaattcagccagcccagcacatccagtcagaaaccagtggatctgccaactactcccaggttgcccacattcccaaatcagatgctttgtactttgatgactgcatgcagcttttggcgcagacattcccgtttgtagatgacaatgaggtttcttcggctacgtttcagtcacttgttcctgatattcccggtcacatcgagagcccagtcttcattgctactaatcaggctcagtcacctgaaacttctgttgctcaggtagcccctgttgatttagacggtatgcaacaggacattgagcaagtttgggaggagctattatccattcctgagttacagtgtcttaatattgaaaatgacaagctggttgagactaccatggttccaagtccagaagccaaactgacagaagttgacaattatcatttttactcatctataccctcaatggaaaaagaagtaggtaactgtagtccacattttcttaatgcttttgaggattccttcagcagcatcctctccacagaagaccccaaccagttgacagtgaactcattaaattcagatgccacagtcaacacagattttggtgatgaattttattctgctttcatagctgagcccagtatcagcaacagcatgccctcacctgctactttaagccattcactctctgaacttctaaatgggcccattgatgtttctgatctatcactttgcaaagctttcaaccaaaaccaccctgaaagcacagcagaattcaatgattctgactccggcatttcactaaacacaagtcccagtgtggcatcaccagaacactcagtggaatcttccagctatggagacacactacttggcctcagtgattctgaagtggaagagctagatagtgcccctggaagtgtcaaacagaatggtcctaaaacaccagtacattcttctggggatatggtacaacccttgtcaccatctcaggggcagagcactcacgtgcatgatgcccaatgtgagaacacaccagagaaagaattgcctgtaagtcctggtcatcggaaaaccccattcacaaaagacaaacattcaagccgcttggaggctcatctcacaagagatgaacttagggcaaaagctctccatatcccattccctgtagaaaaaatcattaacctccctgttgttgacttcaacgaaatgatgtccaaagagcagttcaatgaagctcaacttgcattaattcgggatatacgtaggaggggtaagaataaagtggctgctcagaattgcagaaaaagaaaactggaaaatatagtagaactagagcaagatttagatcatttgaaagatgaaaaagaaaaattgctcaaagaaaaaggagaaaatgacaaaagccttcacctactgaaaaaacaactcagcaccttatatctcgaagttttcagcatgctacgtgatgaagatggaaaaccttattctcctagtgaatactccctgcagcaaacaagagatggcaatgttttccttgttcccaaaagtaagaagccagatgttaagaaaaactagatttaggaggatttgaccttttctgagctagtttttttgtactattatactaaaagctcctactgtgatgtgaaatgctcatactttataagtaattctatgcaaaatcatagccaaaactagtatagaaaataatacgaaactttaaaaagcattggagtgtcagtatgttgaatcagtagtttcactttaactgtaaacaatttcttaggacaccatttgggctagtttctgtgtaagtgtaaatactacaaaaacttatttatactgttcttatgtcatttgttatattcatagatttatatgatgatatgacatctggctaaaaagaaattattgcaaaactaaccactatgtacttttttataaatactgtatggacaaaaaatggcattttttatattaaattgtttagctctggcaaaaaaaaaaaattttaagagctggtactaataaaggattattatgactgttaaattattaaaa

SEQ ID NO: 6 - DNA, 2967 bp, Homo sapiens
ggcccttccggggctgcgcggctcccccgcctcggtgccggcaaaaatgtgcctagtcacggggccgctctcgggggaactgaggtcgccttcgggctgggacccggagccccttcgccgcgccccaagacctccttgagtgcgggctgcgacgcgctcaccccgctgggccgtctgtgggcgcggctttgcgaagtcatccatctctcggatcactctctggcagccttgagctctcttgaaagcccagccccgggacgagggaggagcgccttaagtgcccagcgggctcagaagccccgacgtgtggcggctgagccgggccccgcgcactttctcggccggggaggggttcgggctcgggcacccggagttggcccctcgtaacgccgcgggaaagtgcgggcgagggcagtggactctgaggccggagtcggcggcacccggggcttctagttcggacgcggtgccccctggtggcgctcaccgcgcgcgtggccttggcttccgtgacagcgctcggttggccgtcacagcagccctcggttggccctttcctgctttatagcgtgcaaacctcgccgcgccagggccaagggacaggttggagctgttgatctgttgcgcaattgctattttccccagagcggctttgtctttggatttagcgtttcagaattgcaattccaaaatgtgtaagacgggatattctcttctgtgctgtcaagggacatggatttgattgacatactttggaggcaagatatagatcttggagtaagtcgagaagtatttgacttcagtcagcgacggaaagagtatgagctggaaaaacagaaaaaacttgaaaaggaaagacaagaacaactccaaaaggagcaagagaaagcctttttcgctcagttacaactagatgaagagacaggtgaatttctcccaattcagccagcccagcacatccagtcagaaaccagtggatctgccaactactcccaggttgcccacattcccaaatcagatgctttgtactttgatgactgcatgcagcttttggcgcagacattcccgtttgtagatgacaatgagtcacttgttcctgatattcccggtcacatcgagagcccagtcttcattgctactaatcaggctcagtcacctgaaacttctgttgctcaggtagcccctgttgatttagacggtatgcaacaggacattgagcaagtttgggaggagctattatccattcctgagttacagtgtcttaatattgaaaatgacaagctggttgagactaccatggttccaagtccagaagccaaactgacagaagttgacaattatcatttttactcatctataccctcaatggaaaaagaagtaggtaactgtagtccacattttcttaatgcttttgaggattccttcagcagcatcctctccacagaagaccccaaccagttgacagtgaactcattaaattcagatgccacagtcaacacagattttggtgatgaattttattctgctttcatagctgagcccagtatcagcaacagcatgccctcacctgctactttaagccattcactctctgaacttctaaatgggcccattgatgtttctgatctatcactttgcaaagctttcaaccaaaaccaccctgaaagcacagcagaattcaatgattctgactccggcatttcactaaacacaagtcccagtgtggcatcaccagaacactcagtggaatcttccagctatggagacacactacttggcctcagtgattctgaagtggaagagctagatagtgcccctggaagtgtcaaacagaatggtcctaaaacaccagtacattcttctggggatatggtacaacccttgtcaccatctcaggggcagagcactcacgtgcatgatgcccaatgtgagaacacaccagagaaagaattgcctgtaagtcctggtcatcggaaaaccccattcacaaaagacaaacattcaagccgcttggaggctcatctcacaagagatgaacttagggcaaaagctctccatatcccattccctgtagaaaaaatcattaacctccctgttgttgacttcaacgaaatgatgtccaaagagcagttcaatgaagctcaacttgcattaattcgggatatacgtaggaggggtaagaataaagtggctgctcagaattgcagaaaaagaaaactggaaaatatagtagaactagagcaagatttagatcatttgaaagatgaaaaagaaaaattgctcaaagaaaaaggagaaaatgacaaaagccttcacctactgaaaaaacaactcagcaccttatatctcgaagttttcagcatgctacgtgatgaagatggaaaaccttattctcctagtgaatactccctgcagcaaacaagagatggcaatgttttccttgttcccaaaagtaagaagccagatgttaagaaaaactagatttaggaggatttgaccttttctgagctagtttttttgtactattatactaaaagctcctactgtgatgtgaaatgctcatactttataagtaattctatgcaaaatcatagccaaaactagtatagaaaataatacgaaactttaaaaagcattggagtgtcagtatgttgaatcagtagtttcactttaactgtaaacaatttcttaggacaccatttgggctagtttctgtgtaagtgtaaatactacaaaaacttatttatactgttcttatgtcatttgttatattcatagatttatatgatgatatgacatctggctaaaaagaaattattgcaaaactaaccactatgtacttttttataaatactgtatggacaaaaaatggcattttttatattaaattgtttagctctggcaaaaaaaaaaaattttaagagctggtactaataaaggattattatgactgttaaattattaaaa